European Patent Application EP 4 467 568 A1, published November 27, 2024. Title: ANTIBODY TARGETING CD25, AND PREPARATION METHOD THEREFOR AND USE THEREOF. Applicant: Nona Biosciences [Suzhou] Co., Ltd. The sequence listing filed with the application follows.

SEQUENCE LISTING (218 sequences)

SEQ ID NO: 1 - protein, 25 aa, synthetic construct [sequence omitted]

SEQ ID NO: 2 - protein, 25 aa, synthetic construct
EVQLLESGGGLVQPGGSLRLSCAAS

SEQ ID NO: 3 - protein, 25 aa, synthetic construct
QVQLQQSGPGLVKPSQTLSLTCAVS

SEQ ID NO: 4 - protein, 25 aa, synthetic construct
QVQLQGSGPGLVKPSGTLSLTCAVS

SEQ ID NO: 5 - protein, 25 aa, synthetic construct
QVQLQQSGPGLVKPSQTLSLTCAIS

SEQ ID NO: 6 - protein, 25 aa, synthetic construct
QVQLQESGPGLVKPSGTLSLTCAVS

SEQ ID NO: 7 - protein, 25 aa, synthetic construct
QVQLVESGGGVVQPGRSLRLSCAAS

SEQ ID NO: 8 - protein, 25 aa, synthetic construct
QVQLQESGPGLVKPSETLSLTCTVS

SEQ ID NO: 9 - protein, 25 aa, synthetic construct
QVQLVQSGGGVVQPGRSLRLSCAAS

SEQ ID NO: 10 - protein, 25 aa, synthetic construct [sequence omitted]

SEQ ID NO: 11 - protein, 25 aa, synthetic construct
QVQLVQSGAEVKKPGASLKVSCKAS

SEQ ID NO: 12 - protein, 25 aa, synthetic construct
QVHLVESGGGVVQPGRSLRLSCAAS

SEQ ID NO: 13 - protein, 7 aa, synthetic construct
GGTFSSL

SEQ ID NO: 14 - protein, 7 aa, synthetic construct
GFTFSSY

SEQ ID NO: 15 - protein, 9 aa, synthetic construct
GDRVSNINA

SEQ ID NO: 16 - protein, 8 aa, synthetic construct
DGSISSSN

SEQ ID NO: 17 - protein, 9 aa, synthetic construct
GDSVSNNNA

SEQ ID NO: 18 - protein, 8 aa, synthetic construct
GGSISSSN

SEQ ID NO: 19 - protein, 8 aa, synthetic construct
PGSISSSN

SEQ ID NO: 20 - protein, 7 aa, synthetic construct
GGSIRSY

SEQ ID NO: 21 - protein, 7 aa, synthetic construct
GFTFSNY

SEQ ID NO: 22 - protein, 7 aa, synthetic construct
EFTFSSY

SEQ ID NO: 23 - protein, 7 aa, synthetic construct
GYTFTGY

SEQ ID NO: 24 - protein, 7 aa, synthetic construct
GFTFSKY

SEQ ID NO: 25 - protein, 19 aa, synthetic construct
AISWVRQAPGQGLEWMGGI

SEQ ID NO: 26 - protein, 19 aa, synthetic construct
AMSWVRQAPGKGLEWVSTL

SEQ ID NO: 27 - protein, 19 aa, synthetic construct
AWNWIRQSPSRGLEWLGRT

SEQ ID NO: 28 - protein, 19 aa, synthetic construct
WWNWVRQPPGKGLEWIGEI

SEQ ID NO: 29 - protein, 19 aa, synthetic construct
YWSWVRQPPGKGLEWIGEI

SEQ ID NO: 30 - protein, 19 aa, synthetic construct
YMHWVRQAPGKGLEWVAVI

SEQ ID NO: 31 - protein, 19 aa, synthetic construct
YWSWIRQPPGKGLEWIGYI

SEQ ID NO: 32 - protein, 19 aa, synthetic construct
DMHWVRQAPGKGLEWVAVI

SEQ ID NO: 33 - protein, 19 aa, synthetic construct
AMSWVRQAPGKGLEWVSTI

SEQ ID NO: 34 - protein, 19 aa, synthetic construct
YMHWVRQAPGQGLEWMGWI

SEQ ID NO: 35 - protein, 19 aa, synthetic construct
DMHWVRQAPGKGLEWVAVV

SEQ ID NO: 36 - protein, 19 aa, synthetic construct
WWSWVRQSPGKGLEWIGEI

SEQ ID NO: 37 - protein, 6 aa, synthetic construct
IPIFGT

SEQ ID NO: 38 - protein, 6 aa, synthetic construct
SGRGGS

SEQ ID NO: 39 - protein, 7 aa, synthetic construct
YYRSKWY

SEQ ID NO: 40 - protein, 5 aa, synthetic construct
YHRGS

SEQ ID NO: 41 - protein, 10 aa, synthetic construct
HYRSDRSKWY

SEQ ID NO: 42 - protein, 5 aa, synthetic construct
YHSGS

SEQ ID NO: 43 - protein, 6 aa, synthetic construct
WYDGSN

SEQ ID NO: 44 - protein, 5 aa, synthetic construct
YYSGS

SEQ ID NO: 45 - protein, 6 aa, synthetic construct
WYDGIN

SEQ ID NO: 46 - protein, 6 aa, synthetic construct
SGSGGN

SEQ ID NO: 47 - protein, 6 aa, synthetic construct
NPNSGG

SEQ ID NO: 48 - protein, 6 aa, synthetic construct
NSNSGD

SEQ ID NO: 49 - protein, 6 aa, synthetic construct
WFDGIN

SEQ ID NO: 50 - protein, 6 aa, synthetic construct
NPPSGG

SEQ ID NO: 51 - protein, 6 aa, synthetic construct
NPQSGG

SEQ ID NO: 52 - protein, 41 aa, synthetic construct
ANYAQKFQGRVTITADESTSTAYMELSSLRSEDTAVYYCAR

SEQ ID NO: 53 - protein, 41 aa, synthetic construct
TYYADSVKGRFTISRDNSNNTLYLQMNSLRAEDTAVYYCAK

SEQ ID NO: 54 - protein, 41 aa, synthetic construct
NDYAVSVKSRISINLDTSKDQFSLQLNPVTPEDTAVYYCAR

SEQ ID NO: 55 - protein, 41 aa, synthetic construct
TNYNPSLKSRVTISVDKSKNQFSLKLSSVTAADTAVYYCTH

SEQ ID NO: 56 - protein, 41 aa, synthetic construct
NDYAVSVKSRITINSDTFKNQFSLQLNPVTPEDTAVYYCAR

SEQ ID NO: 57 - protein, 41 aa, synthetic construct
TNYNPSLKSRVTISLDKSKNQFSLKLSSVTAADTAVYYCAR

SEQ ID NO: 58 - protein, 41 aa, synthetic construct
KYYADSVKGRFTISRDNSKNTLYLQMNSLRAEDTAVYYCAG

SEQ ID NO: 59 - protein, 41 aa, synthetic construct
TNYNPSLKSRVTISVDTSKNQFSLKLSSVTAADTAVYYCAR

SEQ ID NO: 60 - protein, 41 aa, synthetic construct
KHYTDSVKGRFTMSRDNFKNTLHLQMNSLRAEDTAIYYCAR

SEQ ID NO: 61 - protein, 41 aa, synthetic construct
TYYADSVEGRFTISRDNSKNTLYLQMNSLRAEDTAVYYCAK

SEQ ID NO: 62 - protein, 41 aa, synthetic construct
TNSAQKFQGRVTMTRDTSINTAYMELSRLRSDDTAVYYCAR

SEQ ID NO: 63 - protein, 41 aa, synthetic construct
KRYAQKFQGRVTVTRDTSISTAYMELSRLRSDDTAVYYCAR

SEQ ID NO: 64 - protein, 41 aa, synthetic construct
KSYIDSVRGRFTISRDNSKSTLYLQMNSLRDDDTAVYYCAR

SEQ ID NO: 65 - protein, 41 aa, synthetic construct
TNYNPSLKSRVTISVDKSKNQFSLKLSSVTAADTAVYYCAR

SEQ ID NO: 66 - protein, 41 aa, synthetic construct
TNYAQKFQGRVTMTRDTSINTAYMELSRLRSDDTAVYYCAR

SEQ ID NO: 67 - protein, 13 aa, synthetic construct
GGSVSGTLVDFDI

SEQ ID NO: 68 - protein, 13 aa, synthetic construct
EGYSSSYYEYFQH

SEQ ID NO: 69 - protein, 8 aa, synthetic construct
DPWEAFDY

SEQ ID NO: 70 - protein, 12 aa, synthetic construct
YYYDSSGYYYGY

SEQ ID NO: 71 - protein, 9 aa, synthetic construct
DWDHDAFDI

SEQ ID NO: 72 - protein, 20 aa, synthetic construct
DRNYGSGNYPHYYHYYGMDV

SEQ ID NO: 73 - protein, 10 aa, synthetic construct
AGKGELPFDY

SEQ ID NO: 74 - protein, 13 aa, synthetic construct
DILTGYSDWFFDL

SEQ ID NO: 75 - protein, 9 aa, synthetic construct
EGAGDAFDI

SEQ ID NO: 76 - protein, 13 aa, synthetic construct
EAYSSSWYEYFQH

SEQ ID NO: 77 - protein, 9 aa, synthetic construct
EGEGDAFDI

SEQ ID NO: 78 - protein, 9 aa, synthetic construct
EGAGDAFDF

SEQ ID NO: 79 - protein, 9 aa, synthetic construct
EGVGDAFDI

SEQ ID NO: 80 - protein, 12 aa, synthetic construct
DRLVAVAGIFDY

SEQ ID NO: 81 - protein, 11 aa, synthetic construct
WGQGTMVTVSS

SEQ ID NO: 82 - protein, 11 aa, synthetic construct
WGQGTLVTVSS

SEQ ID NO: 83 - protein, 11 aa, synthetic construct
WGQGTTVTVSS

SEQ ID NO: 84 - protein, 11 aa, synthetic construct
WGRGTLVTVSS

SEQ ID NO: 85 - protein, 11 aa, synthetic construct
WGQGTMVIVSS

SEQ ID NO: 86 - protein, 11 aa, synthetic construct
WGQGAMVTVSS

SEQ ID NO: 87 - protein, 23 aa, synthetic construct
DIQMTQSPSTLSASVGDRVTITC

SEQ ID NO: 88 - protein, 23 aa, synthetic construct
EIVLTQSPATLSVSPGERATLSC

SEQ ID NO: 89 - protein, 23 aa, synthetic construct
EIVMTQSPATLSVSPGERATLSC

SEQ ID NO: 90 - protein, 23 aa, synthetic construct
DIVMTQSPLSLPVTPGEPASISC

SEQ ID NO: 91 - protein, 23 aa, synthetic construct
DIQMTQSPSSLSASVGDRVTVTC

SEQ ID NO: 92 - protein, 23 aa, synthetic construct
DFQMTQSPSTLSASVGDRVTITC

SEQ ID NO: 93 - protein, 23 aa, synthetic construct
EIVMTQSPATLSVSPGERATFSC

SEQ ID NO: 94 - protein, 11 aa, synthetic construct
RASQSISSWLA

SEQ ID NO: 95 - protein, 11 aa, synthetic construct
RASQSISSNLA

SEQ ID NO: 96 - protein, 11 aa, synthetic construct
RASQSVSSNLA

SEQ ID NO: 97 - protein, 16 aa, synthetic construct
RSSQSLLHRDGYNYVD

SEQ ID NO: 98 - protein, 11 aa, synthetic construct
RASQSISGWLA

SEQ ID NO: 99 - protein, 11 aa, synthetic construct
RASQNISSYLN

SEQ ID NO: 100 - protein, 16 aa, synthetic construct
RSSQSLLHSNGYNYLD

SEQ ID NO: 101 - protein, 16 aa, synthetic construct
RSSQSLLHRDVYNYVD

SEQ ID NO: 102 - protein, 16 aa, synthetic construct
RSSQSLLHRRGYNYVD

SEQ ID NO: 103 - protein, 11 aa, synthetic construct
RASQSFDNWLA

SEQ ID NO: 104 - protein, 11 aa, synthetic construct
RASQSVSDTLA

SEQ ID NO: 105 - protein, 11 aa, synthetic construct
RASQTVSSDLA

SEQ ID NO: 106 - protein, 15 aa, synthetic construct
WYQQKPGKAPKLLIY

SEQ ID NO: 107 - protein, 15 aa, synthetic construct
WYQQKPGQAPRLLIY

SEQ ID NO: 108 - protein, 15 aa, synthetic construct
WYLQKPGQSPQLLIY

SEQ ID NO: 109 - protein, 15 aa, synthetic construct
WYLQRPGQSPQLLIY

SEQ ID NO: 110 - protein, 7 aa, synthetic construct
KASSLES

SEQ ID NO: 111 - protein, 7 aa, synthetic construct
GASTRAT

SEQ ID NO: 112 - protein, 7 aa, synthetic construct
AASTRAT

SEQ ID NO: 113 - protein, 7 aa, synthetic construct
LGSNRAS

SEQ ID NO: 114 - protein, 7 aa, synthetic construct
KASSLET

SEQ ID NO: 115 - protein, 7 aa, synthetic construct
AASSLQS

SEQ ID NO: 116 - protein, 7 aa, synthetic construct
EASSLKS

SEQ ID NO: 117 - protein, 32 aa, synthetic construct
GVPSRFSGSGSGTEFTLTISSLQPDDFATYYC

SEQ ID NO: 118 - protein, 32 aa, synthetic construct
GIPARFSGSGSGTEFTLTISSLQSEDFAVYSC

SEQ ID NO: 119 - protein, 32 aa, synthetic construct
GIPARFSGSGSGTEFTLTISSLQSEDFAVYFC

SEQ ID NO: 120 - protein, 32 aa, synthetic construct
GVPDRFSGSGSGTDFTLKISRVEAEDVGVYYC

SEQ ID NO: 121 - protein, 32 aa, synthetic construct
GVPSRFSGSGSGTDFTLTISSLQPEDFATYYC

SEQ ID NO: 122 - protein, 32 aa, synthetic construct
GIPARFSGSGSGTEFTLTISSLQSEDFAVYYC

SEQ ID NO: 123 - protein, 32 aa, synthetic construct
GVPSRFSGSESGTEFTLTISSLQPDDFATYYC

SEQ ID NO: 124 - protein, 32 aa, synthetic construct
GVPSRFSGSESGTEFTLTITSLQPNDFATYYC

SEQ ID NO: 125 - protein, 32 aa, synthetic construct
GIPARFSGSGSGTEFTLTISSLQSEDFAFYYC

SEQ ID NO: 126 - protein, 9 aa, synthetic construct
QQYNIYPIT

SEQ ID NO: 127 - protein, 9 aa, synthetic construct
QQYNYWPLT

SEQ ID NO: 128 - protein, 9 aa, synthetic construct
QQYNDWSIT

SEQ ID NO: 129 - protein, 9 aa, synthetic construct
MQALQTPLT

SEQ ID NO: 130 - protein, 8 aa, synthetic construct
LQYNGYST

SEQ ID NO: 131 - protein, 9 aa, synthetic construct
QQSYSIPYT

SEQ ID NO: 132 - protein, 9 aa, synthetic construct
MQVLQTPYT

SEQ ID NO: 133 - protein, 8 aa, synthetic construct
QQYNNWIT

SEQ ID NO: 134 - protein, 8 aa, synthetic construct
QQYNSYST

SEQ ID NO: 135 - protein, 8 aa, synthetic construct
HQYNSYST

SEQ ID NO: 136 - protein, 9 aa, synthetic construct
QQSNDWPYT

SEQ ID NO: 137 - protein, 8 aa, synthetic construct
HQYLSYST

SEQ ID NO: 138 - protein, 8 aa, synthetic construct
HQYMSYST

SEQ ID NO: 139 - protein, 9 aa, synthetic construct
LQALQTPLT

SEQ ID NO: 140 - protein, 10 aa, synthetic construct
FGGGTKVEIK

SEQ ID NO: 141 - protein, 10 aa, synthetic construct
FGQGTRLEIK

SEQ ID NO: 142 - protein, 10 aa, synthetic construct
FGQGTKLEIK

SEQ ID NO: 143 - protein, 10 aa, synthetic construct
FGGGTKVEIR

SEQ ID NO: 144 - protein, 10 aa, synthetic construct
FGQGTKVEIK

SEQ ID NO: 145 - protein, 122 aa, synthetic construct
QVQLVQSGAEVKKPGSSVKVSCKASGGTFSSLAISWVRQAPGQGLEWMGGIIPIFGTANYAQKFQGRVTITADESTSTAYMELSSLRSEDTAVYYCARGGSVSGTLVDFDIWGQGTMVTVSS

SEQ ID NO: 146 - protein, 122 aa, synthetic construct
EVQLLESGGGLVQPGGSLRLSCAASGFTFSSYAMSWVRQAPGKGLEWVSTLSGRGGSTYYADSVKGRFTISRDNSNNTLYLQMNSLRAEDTAVYYCAKEGYSSSYYEYFQHWGQGTLVTVSS

SEQ ID NO: 147 - protein, 120 aa, synthetic construct
QVQLQQSGPGLVKPSQTLSLTCAVSGDRVSNINAAWNWIRQSPSRGLEWLGRTYYRSKWYNDYAVSVKSRISINLDTSKDQFSLQLNPVTPEDTAVYYCARDPWEAFDYWGQGTLVTVSS

SEQ ID NO: 148 - protein, 121 aa, synthetic construct
QVQLQGSGPGLVKPSGTLSLTCAVSDGSISSSNWWNWVRQPPGKGLEWIGEIYHRGSTNYNPSLKSRVTISVDKSKNQFSLKLSSVTAADTAVYYCTHYYYDSSGYYYGYWGQGTLVTVSS

SEQ ID NO: 149 - protein, 124 aa, synthetic construct
QVQLQQSGPGLVKPSQTLSLTCAISGDSVSNNNAAWNWIRQSPSRGLEWLGRTHYRSDRSKWYNDYAVSVKSRITINSDTFKNQFSLQLNPVTPEDTAVYYCARDWDHDAFDIWGQGTMVTVSS

SEQ ID NO: 150 - protein, 129 aa, synthetic construct
QVQLQESGPGLVKPSGTLSLTCAVSGGSISSSNYWSWVRQPPGKGLEWIGEIYHSGSTNYNPSLKSRVTISLDKSKNQFSLKLSSVTAADTAVYYCARDRNYGSGNYPHYYHYYGMDVWGQGTTVTVSS

SEQ ID NO: 151 - protein, 119 aa, synthetic construct
QVQLVESGGGVVQPGRSLRLSCAASGFTFSSYYMHWVRQAPGKGLEWVAVIWYDGSNKYYADSVKGRFTISRDNSKNTLYLQMNSLRAEDTAVYYCAGAGKGELPFDYWGQGTLVTVSS

SEQ ID NO: 152 - protein, 121 aa, synthetic construct
QVQLQGSGPGLVKPSGTLSLTCAVSPGSISSSNWWNWVRQPPGKGLEWIGEIYHRGSTNYNPSLKSRVTISVDKSKNQFSLKLSSVTAADTAVYYCTHYYYDSSGYYYGYWGQGTLVTVSS

SEQ ID NO: 153 - protein, 121 aa, synthetic construct
QVQLQESGPGLVKPSETLSLTCTVSGGSIRSYYWSWIRQPPGKGLEWIGYIYYSGSTNYNPSLKSRVTISVDTSKNQFSLKLSSVTAADTAVYYCARDILTGYSDWFFDLWGRGTLVTVSS

SEQ ID NO: 154 - protein, 118 aa, synthetic construct
QVQLVQSGGGVVQPGRSLRLSCAASGFTFSNYDMHWVRQAPGKGLEWVAVIWYDGINKHYTDSVKGRFTMSRDNFKNTLHLQMNSLRAEDTAIYYCAREGAGDAFDIWGQGTMVTVSS

SEQ ID NO: 155 - protein, 122 aa, synthetic construct
EVQLLESGGGLVQPGGSLRLSCAASEFTFSSYAMSWVRQAPGKGLEWVSTISGSGGNTYYADSVEGRFTISRDNSKNTLYLQMNSLRAEDTAVYYCAKEAYSSSWYEYFQHWGQGTLVTVSS

SEQ ID NO: 156 - protein, 118 aa, synthetic construct
QVQLVQSGAEVKKPGASVKVSCKASGYTFTGYYMHWVRQAPGQGLEWMGWINPNSGGTNSAQKFQGRVTMTRDTSINTAYMELSRLRSDDTAVYYCAREGEGDAFDIWGQGTMVTVSS

SEQ ID NO: 157 - protein, 118 aa, synthetic construct
QVQLVQSGAEVKKPGASLKVSCKASGYTFTGYYMHWVRQAPGQGLEWMGWINSNSGDKRYAQKFQGRVTVTRDTSISTAYMELSRLRSDDTAVYYCAREGAGDAFDFWGQGTMVIVSS

SEQ ID NO: 158 - protein, 118 aa, synthetic construct
QVHLVESGGGVVQPGRSLRLSCAASGFTFSKYDMHWVRQAPGKGLEWVAVVWFDGINKSYIDSVRGRFTISRDNSKSTLYLQMNSLRDDDTAVYYCAREGVGDAFDIWGQGAMVTVSS

SEQ ID NO: 159 - protein, 121 aa, synthetic construct
QVQLQESGPGLVKPSGTLSLTCAVSGGSISSSNWWSWVRQSPGKGLEWIGEIYHSGSTNYNPSLKSRVTISVDKSKNQFSLKLSSVTAADTAVYYCARDRLVAVAGIFDYWGQGTLVTVSS

SEQ ID NO: 160 - protein, 118 aa, synthetic construct
QVQLVQSGAEVKKPGASVKVSCKASGYTFTGYYMHWVRQAPGQGLEWMGWINPPSGGTNYAQKFQGRVTMTRDTSINTAYMELSRLRSDDTAVYYCAREGEGDAFDIWGQGTMVTVSS

SEQ ID NO: 161 - protein, 118 aa, synthetic construct
QVQLVQSGAEVKKPGASVKVSCKASGYTFTGYYMHWVRQAPGQGLEWMGWINPQSGGTNYAQKFQGRVTMTRDTSINTAYMELSRLRSDDTAVYYCAREGEGDAFDIWGQGTMVTVSS

SEQ ID NO: 162 - protein, 107 aa, synthetic construct
DIQMTQSPSTLSASVGDRVTITCRASQSISSWLAWYQQKPGKAPKLLIYKASSLESGVPSRFSGSGSGTEFTLTISSLQPDDFATYYCQQYNIYPITFGGGTKVEIK

SEQ ID NO: 163 - protein, 107 aa, synthetic construct
EIVLTQSPATLSVSPGERATLSCRASQSISSNLAWYQQKPGQAPRLLIYGASTRATGIPARFSGSGSGTEFTLTISSLQSEDFAVYSCQQYNYWPLTFGGGTKVEIK

SEQ ID NO: 164 - protein, 107 aa, synthetic construct
EIVMTQSPATLSVSPGERATLSCRASQSVSSNLAWYQQKPGQAPRLLIYAASTRATGIPARFSGSGSGTEFTLTISSLQSEDFAVYFCQQYNDWSITFGQGTRLEIK

SEQ ID NO: 165 - protein, 112 aa, synthetic construct
DIVMTQSPLSLPVTPGEPASISCRSSQSLLHRDGYNYVDWYLQKPGQSPQLLIYLGSNRASGVPDRFSGSGSGTDFTLKISRVEAEDVGVYYCMQALQTPLTFGGGTKVEIK

SEQ ID NO: 166 - protein, 106 aa, synthetic construct
DIQMTQSPSTLSASVGDRVTITCRASQSISGWLAWYQQKPGKAPKLLIYKASSLETGVPSRFSGSGSGTEFTLTISSLQPDDFATYYCLQYNGYSTFGGGTKVEIK

SEQ ID NO: 167 - protein, 107 aa, synthetic construct
DIQMTQSPSSLSASVGDRVTVTCRASQNISSYLNWYQQKPGKAPKLLIYAASSLQSGVPSRFSGSGSGTDFTLTISSLQPEDFATYYCQQSYSIPYTFGQGTKLEIK

SEQ ID NO: 168 - protein, 112 aa, synthetic construct
DIVMTQSPLSLPVTPGEPASISCRSSQSLLHSNGYNYLDWYLQRPGQSPQLLIYLGSNRASGVPDRFSGSGSGTDFTLKISRVEAEDVGVYYCMQVLQTPYTFGQGTKLEIK

SEQ ID NO: 169 - protein, 112 aa, synthetic construct
DIVMTQSPLSLPVTPGEPASISCRSSQSLLHRDVYNYVDWYLQKPGQSPQLLIYLGSNRASGVPDRFSGSGSGTDFTLKISRVEAEDVGVYYCMQALQTPLTFGGGTKVEIK

SEQ ID NO: 170 - protein, 112 aa, synthetic construct
DIVMTQSPLSLPVTPGEPASISCRSSQSLLHRRGYNYVDWYLQKPGQSPQLLIYLGSNRASGVPDRFSGSGSGTDFTLKISRVEAEDVGVYYCMQALQTPLTFGGGTKVEIK

SEQ ID NO: 171 - protein, 106 aa, synthetic construct
EIVMTQSPATLSVSPGERATLSCRASQSVSSNLAWYQQKPGQAPRLLIYGASTRATGIPARFSGSGSGTEFTLTISSLQSEDFAVYYCQQYNNWITFGQGTRLEIK

SEQ ID NO: 172 - protein, 106 aa, synthetic construct
DIQMTQSPSTLSASVGDRVTITCRASQSFDNWLAWYQQKPGKAPKLLIYKASSLESGVPSRFSGSGSGTEFTLTISSLQPDDFATYYCQQYNSYSTFGQGTRLEIK

SEQ ID NO: 173 - protein, 107 aa, synthetic construct
EIVMTQSPATLSVSPGERATLSCRASQSVSDTLAWYQQKPGQAPRLLIYGASTRATGIPARFSGSGSGTEFTLTISSLQSEDFAVYYCQQYNYWPLTFGGGTKVEIR

SEQ ID NO: 174 - protein, 106 aa, synthetic construct
DFQMTQSPSTLSASVGDRVTITCRASQSISSWLAWYQQKPGKAPKLLIYEASSLKSGVPSRFSGSESGTEFTLTISSLQPDDFATYYCHQYNSYSTFGQGTKVEIK

SEQ ID NO: 175 - protein, 106 aa, synthetic construct
DIQMTQSPSTLSASVGDRVTITCRASQSISSWLAWYQQKPGKAPKLLIYKASSLESGVPSRFSGSESGTEFTLTISSLQPDDFATYYCQQYNSYSTFGQGTKVEIK

SEQ ID NO: 176 - protein, 106 aa, synthetic construct
DIQMTQSPSTLSASVGDRVTITCRASQSISSWLAWYQQKPGKAPKLLIYKASSLESGVPSRFSGSESGTEFTLTITSLQPNDFATYYCQQYNSYSTFGQGTRLEIK

SEQ ID NO: 177 - protein, 107 aa, synthetic construct
EIVMTQSPATLSVSPGERATFSCRASQTVSSDLAWYQQKPGQAPRLLIYGASTRATGIPARFSGSGSGTEFTLTISSLQSEDFAFYYCQQSNDWPYTFGQGTKLEIK

SEQ ID NO: 178 - protein, 106 aa, synthetic construct
DFQMTQSPSTLSASVGDRVTITCRASQSISSWLAWYQQKPGKAPKLLIYEASSLKSGVPSRFSGSESGTEFTLTISSLQPDDFATYYCHQYLSYSTFGQGTKVEIK

SEQ ID NO: 179 - protein, 106 aa, synthetic construct
DFQMTQSPSTLSASVGDRVTITCRASQSISSWLAWYQQKPGKAPKLLIYEASSLKSGVPSRFSGSESGTEFTLTISSLQPDDFATYYCHQYMSYSTFGQGTKVEIK

SEQ ID NO: 180 - protein, 112 aa, synthetic construct
DIVMTQSPLSLPVTPGEPASISCRSSQSLLHRDVYNYVDWYLQKPGQSPQLLIYLGSNRASGVPDRFSGSGSGTDFTLKISRVEAEDVGVYYCLQALQTPLTFGGGTKVEIK

SEQ ID NO: 181 - protein, 452 aa, synthetic construct
QVQLVQSGAEVKKPGSSVKVSCKASGGTFSSLAISWVRQAPGQGLEWMGGIIPIFGTANYAQKFQGRVTITADESTSTAYMELSSLRSEDTAVYYCARGGSVSGTLVDFDIWGQGTMVTVSSASTKGPSVFPLAPSSKSTSGGTAALGCLVKDYFPEPVTVSWNSGALTSGVHTFPAVLQSSGLYSLSSVVTVPSSSLGTQTYICNVNHKPSNTKVDKKVEPKSCDKTHTCPPCPAPELLGGPSVFLFPPKPKDTLMISRTPEVTCVVVDVSHEDPEVKFNWYVDGVEVHNAKTKPREEQYNSTYRVVSVLTVLHQDWLNGKEYKCKVSNKALPAPIEKTISKAKGQPREPQVYTLPPSREEMTKNQVSLTCLVKGFYPSDIAVEWESNGQPENNYKTTPPVLDSDGSFFLYSKLTVDKSRWQQGNVFSCSVMHEALHNHYTQKSLSLSPGK

SEQ ID NO: 182 - protein, 452 aa, synthetic construct
EVQLLESGGGLVQPGGSLRLSCAASGFTFSSYAMSWVRQAPGKGLEWVSTLSGRGGSTYYADSVKGRFTISRDNSNNTLYLQMNSLRAEDTAVYYCAKEGYSSSYYEYFQHWGQGTLVTVSSASTKGPSVFPLAPSSKSTSGGTAALGCLVKDYFPEPVTVSWNSGALTSGVHTFPAVLQSSGLYSLSSVVTVPSSSLGTQTYICNVNHKPSNTKVDKKVEPKSCDKTHTCPPCPAPELLGGPDVFLFPPKPKDTLMISRTPEVTCVVVDVSHEDPEVKFNWYVDGVEVHNAKTKPREEQYNSTYRVVSVLTVLHQDWLNGKEYKCKVSNKALPAPEEKTISKAKGQPREPQVYTLPPSREEMTKNQVSLTCLVKGFYPSDIAVEWESNGQPENNYKTTPPVLDSDGSFFLYSKLTVDKSRWQQGNVFSCSVMHEALHNHYTQKSLSLSPGK

SEQ ID NO: 183 - protein, 450 aa, synthetic construct
QVQLQQSGPGLVKPSQTLSLTCAVSGDRVSNINAAWNWIRQSPSRGLEWLGRTYYRSKWYNDYAVSVKSRISINLDTSKDQFSLQLNPVTPEDTAVYYCARDPWEAFDYWGQGTLVTVSSASTKGPSVFPLAPSSKSTSGGTAALGCLVKDYFPEPVTVSWNSGALTSGVHTFPAVLQSSGLYSLSSVVTVPSSSLGTQTYICNVNHKPSNTKVDKKVEPKSCDKTHTCPPCPAPELLGGPDVFLFPPKPKDTLMISRTPEVTCVVVDVSHEDPEVKFNWYVDGVEVHNAKTKPREEQYNSTYRVVSVLTVLHQDWLNGKEYKCKVSNKALPAPEEKTISKAKGQPREPQVYTLPPSREEMTKNQVSLTCLVKGFYPSDIAVEWESNGQPENNYKTTPPVLDSDGSFFLYSKLTVDKSRWQQGNVFSCSVMHEALHNHYTQKSLSLSPGK

SEQ ID NO: 184 - protein, 451 aa, synthetic construct
QVQLQGSGPGLVKPSGTLSLTCAVSDGSISSSNWWNWVRQPPGKGLEWIGEIYHRGSTNYNPSLKSRVTISVDKSKNQFSLKLSSVTAADTAVYYCTHYYYDSSGYYYGYWGQGTLVTVSSASTKGPSVFPLAPSSKSTSGGTAALGCLVKDYFPEPVTVSWNSGALTSGVHTFPAVLQSSGLYSLSSVVTVPSSSLGTQTYICNVNHKPSNTKVDKKVEPKSCDKTHTCPPCPAPELLGGPDVFLFPPKPKDTLMISRTPEVTCVVVDVSHEDPEVKFNWYVDGVEVHNAKTKPREEQYNSTYRVVSVLTVLHQDWLNGKEYKCKVSNKALPAPEEKTISKAKGQPREPQVYTLPPSREEMTKNQVSLTCLVKGFYPSDIAVEWESNGQPENNYKTTPPVLDSDGSFFLYSKLTVDKSRWQQGNVFSCSVMHEALHNHYTQKSLSLSPGK

SEQ ID NO: 185 - protein, 454 aa, synthetic construct
QVQLQQSGPGLVKPSQTLSLTCAISGDSVSNNNAAWNWIRQSPSRGLEWLGRTHYRSDRSKWYNDYAVSVKSRITINSDTFKNQFSLQLNPVTPEDTAVYYCARDWDHDAFDIWGQGTMVTVSSASTKGPSVFPLAPSSKSTSGGTAALGCLVKDYFPEPVTVSWNSGALTSGVHTFPAVLQSSGLYSLSSVVTVPSSSLGTQTYICNVNHKPSNTKVDKKVEPKSCDKTHTCPPCPAPELLGGPDVFLFPPKPKDTLMISRTPEVTCVVVDVSHEDPEVKFNWYVDGVEVHNAKTKPREEQYNSTYRVVSVLTVLHQDWLNGKEYKCKVSNKALPAPEEKTISKAKGQPREPQVYTLPPSREEMTKNQVSLTCLVKGFYPSDIAVEWESNGQPENNYKTTPPVLDSDGSFFLYSKLTVDKSRWQQGNVFSCSVMHEALHNHYTQKSLSLSPGK

SEQ ID NO: 186 - protein, 459 aa, synthetic construct
QVQLQESGPGLVKPSGTLSLTCAVSGGSISSSNYWSWVRQPPGKGLEWIGEIYHSGSTNYNPSLKSRVTISLDKSKNQFSLKLSSVTAADTAVYYCARDRNYGSGNYPHYYHYYGMDVWGQGTTVTVSSASTKGPSVFPLAPSSKSTSGGTAALGCLVKDYFPEPVTVSWNSGALTSGVHTFPAVLQSSGLYSLSSVVTVPSSSLGTQTYICNVNHKPSNTKVDKKVEPKSCDKTHTCPPCPAPELLGGPSVFLFPPKPKDTLMISRTPEVTCVVVDVSHEDPEVKFNWYVDGVEVHNAKTKPREEQYNSTYRVVSVLTVLHQDWLNGKEYKCKVSNKALPAPIEKTISKAKGQPREPQVYTLPPSREEMTKNQVSLTCLVKGFYPSDIAVEWESNGQPENNYKTTPPVLDSDGSFFLYSKLTVDKSRWQQGNVFSCSVMHEALHNHYTQKSLSLSPGK

SEQ ID NO: 187 - protein, 449 aa, synthetic construct
QVQLVESGGGVVQPGRSLRLSCAASGFTFSSYYMHWVRQAPGKGLEWVAVIWYDGSNKYYADSVKGRFTISRDNSKNTLYLQMNSLRAEDTAVYYCAGAGKGELPFDYWGQGTLVTVSSASTKGPSVFPLAPSSKSTSGGTAALGCLVKDYFPEPVTVSWNSGALTSGVHTFPAVLQSSGLYSLSSVVTVPSSSLGTQTYICNVNHKPSNTKVDKKVEPKSCDKTHTCPPCPAPELLGGPDVFLFPPKPKDTLMISRTPEVTCVVVDVSHEDPEVKFNWYVDGVEVHNAKTKPREEQYNSTYRVVSVLTVLHQDWLNGKEYKCKVSNKALPAPEEKTISKAKGQPREPQVYTLPPSREEMTKNQVSLTCLVKGFYPSDIAVEWESNGQPENNYKTTPPVLDSDGSFFLYSKLTVDKSRWQQGNVFSCSVMHEALHNHYTQKSLSLSPGK

SEQ ID NO: 188 - protein, 451 aa, synthetic construct
QVQLQGSGPGLVKPSGTLSLTCAVSPGSISSSNWWNWVRQPPGKGLEWIGEIYHRGSTNYNPSLKSRVTISVDKSKNQFSLKLSSVTAADTAVYYCTHYYYDSSGYYYGYWGQGTLVTVSSASTKGPSVFPLAPSSKSTSGGTAALGCLVKDYFPEPVTVSWNSGALTSGVHTFPAVLQSSGLYSLSSVVTVPSSSLGTQTYICNVNHKPSNTKVDKKVEPKSCDKTHTCPPCPAPELLGGPSVFLFPPKPKDTLMISRTPEVTCVVVDVSHEDPEVKFNWYVDGVEVHNAKTKPREEQYNSTYRVVSVLTVLHQDWLNGKEYKCKVSNKALPAPIEKTISKAKGQPREPQVYTLPPSREEMTKNQVSLTCLVKGFYPSDIAVEWESNGQPENNYKTTPPVLDSDGSFFLYSKLTVDKSRWQQGNVFSCSVMHEALHNHYTQKSLSLSPGK

SEQ ID NO: 189 - protein, 451 aa, synthetic construct
QVQLQESGPGLVKPSETLSLTCTVSGGSIRSYYWSWIRQPPGKGLEWIGYIYYSGSTNYNPSLKSRVTISVDTSKNQFSLKLSSVTAADTAVYYCARDILTGYSDWFFDLWGRGTLVTVSSASTKGPSVFPLAPSSKSTSGGTAALGCLVKDYFPEPVTVSWNSGALTSGVHTFPAVLQSSGLYSLSSVVTVPSSSLGTQTYICNVNHKPSNTKVDKKVEPKSCDKTHTCPPCPAPELLGGPSVFLFPPKPKDTLMISRTPEVTCVVVDVSHEDPEVKFNWYVDGVEVHNAKTKPREEQYNSTYRVVSVLTVLHQDWLNGKEYKCKVSNKALPAPIEKTISKAKGQPREPQVYTLPPSREEMTKNQVSLTCLVKGFYPSDIAVEWESNGQPENNYKTTPPVLDSDGSFFLYSKLTVDKSRWQQGNVFSCSVMHEALHNHYTQKSLSLSPGK

SEQ ID NO: 190 - protein, 448 aa, synthetic construct
QVQLVQSGGGVVQPGRSLRLSCAASGFTFSNYDMHWVRQAPGKGLEWVAVIWYDGINKHYTDSVKGRFTMSRDNFKNTLHLQMNSLRAEDTAIYYCAREGAGDAFDIWGQGTMVTVSSASTKGPSVFPLAPSSKSTSGGTAALGCLVKDYFPEPVTVSWNSGALTSGVHTFPAVLQSSGLYSLSSVVTVPSSSLGTQTYICNVNHKPSNTKVDKKVEPKSCDKTHTCPPCPAPELLGGPSVFLFPPKPKDTLMISRTPEVTCVVVDVSHEDPEVKFNWYVDGVEVHNAKTKPREEQYNSTYRVVSVLTVLHQDWLNGKEYKCKVSNKALPAPIEKTISKAKGQPREPQVYTLPPSREEMTKNQVSLTCLVKGFYPSDIAVEWESNGQPENNYKTTPPVLDSDGSFFLYSKLTVDKSRWQQGNVFSCSVMHEALHNHYTQKSLSLSPGK

SEQ ID NO: 191 - protein, 452 aa, synthetic construct
EVQLLESGGGLVQPGGSLRLSCAASEFTFSSYAMSWVRQAPGKGLEWVSTISGSGGNTYYADSVEGRFTISRDNSKNTLYLQMNSLRAEDTAVYYCAKEAYSSSWYEYFQHWGQGTLVTVSSASTKGPSVFPLAPSSKSTSGGTAALGCLVKDYFPEPVTVSWNSGALTSGVHTFPAVLQSSGLYSLSSVVTVPSSSLGTQTYICNVNHKPSNTKVDKKVEPKSCDKTHTCPPCPAPELLGGPSVFLFPPKPKDTLMISRTPEVTCVVVDVSHEDPEVKFNWYVDGVEVHNAKTKPREEQYNSTYRVVSVLTVLHQDWLNGKEYKCKVSNKALPAPIEKTISKAKGQPREPQVYTLPPSREEMTKNQVSLTCLVKGFYPSDIAVEWESNGQPENNYKTTPPVLDSDGSFFLYSKLTVDKSRWQQGNVFSCSVMHEALHNHYTQKSLSLSPGK

SEQ ID NO: 192 - protein, 448 aa, synthetic construct
QVQLVQSGAEVKKPGASVKVSCKASGYTFTGYYMHWVRQAPGQGLEWMGWINPNSGGTNSAQKFQGRVTMTRDTSINTAYMELSRLRSDDTAVYYCAREGEGDAFDIWGQGTMVTVSSASTKGPSVFPLAPSSKSTSGGTAALGCLVKDYFPEPVTVSWNSGALTSGVHTFPAVLQSSGLYSLSSVVTVPSSSLGTQTYICNVNHKPSNTKVDKKVEPKSCDKTHTCPPCPAPELLGGPSVFLFPPKPKDTLMISRTPEVTCVVVDVSHEDPEVKFNWYVDGVEVHNAKTKPREEQYNSTYRVVSVLTVLHQDWLNGKEYKCKVSNKALPAPIEKTISKAKGQPREPQVYTLPPSREEMTKNQVSLTCLVKGFYPSDIAVEWESNGQPENNYKTTPPVLDSDGSFFLYSKLTVDKSRWQQGNVFSCSVMHEALHNHYTQKSLSLSPGK

SEQ ID NO: 193 - protein, 448 aa, synthetic construct
QVQLVQSGAEVKKPGASLKVSCKASGYTFTGYYMHWVRQAPGQGLEWMGWINSNSGDKRYAQKFQGRVTVTRDTSISTAYMELSRLRSDDTAVYYCAREGAGDAFDFWGQGTMVIVSSASTKGPSVFPLAPSSKSTSGGTAALGCLVKDYFPEPVTVSWNSGALTSGVHTFPAVLQSSGLYSLSSVVTVPSSSLGTQTYICNVNHKPSNTKVDKKVEPKSCDKTHTCPPCPAPELLGGPSVFLFPPKPKDTLMISRTPEVTCVVVDVSHEDPEVKFNWYVDGVEVHNAKTKPREEQYNSTYRVVSVLTVLHQDWLNGKEYKCKVSNKALPAPIEKTISKAKGQPREPQVYTLPPSREEMTKNQVSLTCLVKGFYPSDIAVEWESNGQPENNYKTTPPVLDSDGSFFLYSKLTVDKSRWQQGNVFSCSVMHEALHNHYTQKSLSLSPGK

SEQ ID NO: 194 - protein, 448 aa, synthetic construct
QVHLVESGGGVVQPGRSLRLSCAASGFTFSKYDMHWVRQAPGKGLEWVAVVWFDGINKSYIDSVRGRFTISRDNSKSTLYLQMNSLRDDDTAVYYCAREGVGDAFDIWGQGAMVTVSSASTKGPSVFPLAPSSKSTSGGTAALGCLVKDYFPEPVTVSWNSGALTSGVHTFPAVLQSSGLYSLSSVVTVPSSSLGTQTYICNVNHKPSNTKVDKKVEPKSCDKTHTCPPCPAPELLGGPSVFLFPPKPKDTLMISRTPEVTCVVVDVSHEDPEVKFNWYVDGVEVHNAKTKPREEQYNSTYRVVSVLTVLHQDWLNGKEYKCKVSNKALPAPIEKTISKAKGQPREPQVYTLPPSREEMTKNQVSLTCLVKGFYPSDIAVEWESNGQPENNYKTTPPVLDSDGSFFLYSKLTVDKSRWQQGNVFSCSVMHEALHNHYTQKSLSLSPGK

SEQ ID NO: 195 - protein, 451 aa, synthetic construct
QVQLQESGPGLVKPSGTLSLTCAVSGGSISSSNWWSWVRQSPGKGLEWIGEIYHSGSTNYNPSLKSRVTISVDKSKNQFSLKLSSVTAADTAVYYCARDRLVAVAGIFDYWGQGTLVTVSSASTKGPSVFPLAPSSKSTSGGTAALGCLVKDYFPEPVTVSWNSGALTSGVHTFPAVLQSSGLYSLSSVVTVPSSSLGTQTYICNVNHKPSNTKVDKKVEPKSCDKTHTCPPCPAPELLGGPSVFLFPPKPKDTLMISRTPEVTCVVVDVSHEDPEVKFNWYVDGVEVHNAKTKPREEQYNSTYRVVSVLTVLHQDWLNGKEYKCKVSNKALPAPIEKTISKAKGQPREPQVYTLPPSREEMTKNQVSLTCLVKGFYPSDIAVEWESNGQPENNYKTTPPVLDSDGSFFLYSKLTVDKSRWQQGNVFSCSVMHEALHNHYTQKSLSLSPGK

SEQ ID NO: 196 - protein, 448 aa, synthetic construct
QVQLVQSGAEVKKPGASVKVSCKASGYTFTGYYMHWVRQAPGQGLEWMGWINPPSGGTNYAQKFQGRVTMTRDTSINTAYMELSRLRSDDTAVYYCAREGEGDAFDIWGQGTMVTVSSASTKGPSVFPLAPSSKSTSGGTAALGCLVKDYFPEPVTVSWNSGALTSGVHTFPAVLQSSGLYSLSSVVTVPSSSLGTQTYICNVNHKPSNTKVDKKVEPKSCDKTHTCPPCPAPELLGGPSVFLFPPKPKDTLMISRTPEVTCVVVDVSHEDPEVKFNWYVDGVEVHNAKTKPREEQYNSTYRVVSVLTVLHQDWLNGKEYKCKVSNKALPAPIEKTISKAKGQPREPQVYTLPPSREEMTKNQVSLTCLVKGFYPSDIAVEWESNGQPENNYKTTPPVLDSDGSFFLYSKLTVDKSRWQQGNVFSCSVMHEALHNHYTQKSLSLSPGK

SEQ ID NO: 197 - protein, 448 aa, synthetic construct
QVQLVQSGAEVKKPGASVKVSCKASGYTFTGYYMHWVRQAPGQGLEWMGWINPQSGGTNYAQKFQGRVTMTRDTSINTAYMELSRLRSDDTAVYYCAREGEGDAFDIWGQGTMVTVSSASTKGPSVFPLAPSSKSTSGGTAALGCLVKDYFPEPVTVSWNSGALTSGVHTFPAVLQSSGLYSLSSVVTVPSSSLGTQTYICNVNHKPSNTKVDKKVEPKSCDKTHTCPPCPAPELLGGPSVFLFPPKPKDTLMISRTPEVTCVVVDVSHEDPEVKFNWYVDGVEVHNAKTKPREEQYNSTYRVVSVLTVLHQDWLNGKEYKCKVSNKALPAPIEKTISKAKGQPREPQVYTLPPSREEMTKNQVSLTCLVKGFYPSDIAVEWESNGQPENNYKTTPPVLDSDGSFFLYSKLTVDKSRWQQGNVFSCSVMHEALHNHYTQKSLSLSPGK

SEQ ID NO: 198 - protein, 214 aa, synthetic construct
DIQMTQSPSTLSASVGDRVTITCRASQSISSWLAWYQQKPGKAPKLLIYKASSLESGVPSRFSGSGSGTEFTLTISSLQPDDFATYYCQQYNIYPITFGGGTKVEIKRTVAAPSVFIFPPSDEQLKSGTASVVCLLNNFYPREAKVQWKVDNALQSGNSQESVTEQDSKDSTYSLSSTLTLSKADYEKHKVYACEVTHQGLSSPVTKSFNRGEC

SEQ ID NO: 199 - protein, 214 aa, synthetic construct
EIVLTQSPATLSVSPGERATLSCRASQSISSNLAWYQQKPGQAPRLLIYGASTRATGIPARFSGSGSGTEFTLTISSLQSEDFAVYSCQQYNYWPLTFGGGTKVEIKRTVAAPSVFIFPPSDEQLKSGTASVVCLLNNFYPREAKVQWKVDNALQSGNSQESVTEQDSKDSTYSLSSTLTLSKADYEKHKVYACEVTHQGLSSPVTKSFNRGEC

SEQ ID NO: 200 - protein, 214 aa, synthetic construct
EIVMTQSPATLSVSPGERATLSCRASQSVSSNLAWYQQKPGQAPRLLIYAASTRATGIPARFSGSGSGTEFTLTISSLQSEDFAVYFCQQYNDWSITFGQGTRLEIKRTVAAPSVFIFPPSDEQLKSGTASVVCLLNNFYPREAKVQWKVDNALQSGNSQESVTEQDSKDSTYSLSSTLTLSKADYEKHKVYACEVTHQGLSSPVTKSFNRGEC

SEQ ID NO: 201 - protein, 219 aa, synthetic construct
DIVMTQSPLSLPVTPGEPASISCRSSQSLLHRDGYNYVDWYLQKPGQSPQLLIYLGSNRASGVPDRFSGSGSGTDFTLKISRVEAEDVGVYYCMQALQTPLTFGGGTKVEIKRTVAAPSVFIFPPSDEQLKSGTASVVCLLNNFYPREAKVQWKVDNALQSGNSQESVTEQDSKDSTYSLSSTLTLSKADYEKHKVYACEVTHQGLSSPVTKSFNRGEC

SEQ ID NO: 202 - protein, 213 aa, synthetic construct
DIQMTQSPSTLSASVGDRVTITCRASQSISGWLAWYQQKPGKAPKLLIYKASSLETGVPSRFSGSGSGTEFTLTISSLQPDDFATYYCLQYNGYSTFGGGTKVEIKRTVAAPSVFIFPPSDEQLKSGTASVVCLLNNFYPREAKVQWKVDNALQSGNSQESVTEQDSKDSTYSLSSTLTLSKADYEKHKVYACEVTHQGLSSPVTKSFNRGEC

SEQ ID NO: 203 - protein, 214 aa, synthetic construct
DIQMTQSPSSLSASVGDRVTVTCRASQNISSYLNWYQQKPGKAPKLLIYAASSLQSGVPSRFSGSGSGTDFTLTISSLQPEDFATYYCQQSYSIPYTFGQGTKLEIKRTVAAPSVFIFPPSDEQLKSGTASVVCLLNNFYPREAKVQWKVDNALQSGNSQESVTEQDSKDSTYSLSSTLTLSKADYEKHKVYACEVTHQGLSSPVTKSFNRGEC

SEQ ID NO: 204 - protein, 219 aa, synthetic construct
DIVMTQSPLSLPVTPGEPASISCRSSQSLLHSNGYNYLDWYLQRPGQSPQLLIYLGSNRASGVPDRFSGSGSGTDFTLKISRVEAEDVGVYYCMQVLQTPYTFGQGTKLEIKRTVAAPSVFIFPPSDEQLKSGTASVVCLLNNFYPREAKVQWKVDNALQSGNSQESVTEQDSKDSTYSLSSTLTLSKADYEKHKVYACEVTHQGLSSPVTKSFNRGEC

SEQ ID NO: 205 - protein, 219 aa, synthetic construct
DIVMTQSPLSLPVTPGEPASISCRSSQSLLHRDVYNYVDWYLQKPGQSPQLLIYLGSNRASGVPDRFSGSGSGTDFTLKISRVEAEDVGVYYCMQALQTPLTFGGGTKVEIKRTVAAPSVFIFPPSDEQLKSGTASVVCLLNNFYPREAKVQWKVDNALQSGNSQESVTEQDSKDSTYSLSSTLTLSKADYEKHKVYACEVTHQGLSSPVTKSFNRGEC

SEQ ID NO: 206 - protein, 219 aa, synthetic construct
DIVMTQSPLSLPVTPGEPASISCRSSQSLLHRRGYNYVDWYLQKPGQSPQLLIYLGSNRASGVPDRFSGSGSGTDFTLKISRVEAEDVGVYYCMQALQTPLTFGGGTKVEIKRTVAAPSVFIFPPSDEQLKSGTASVVCLLNNFYPREAKVQWKVDNALQSGNSQESVTEQDSKDSTYSLSSTLTLSKADYEKHKVYACEVTHQGLSSPVTKSFNRGEC

SEQ ID NO: 207 - protein, 213 aa, synthetic construct
EIVMTQSPATLSVSPGERATLSCRASQSVSSNLAWYQQKPGQAPRLLIYGASTRATGIPARFSGSGSGTEFTLTISSLQSEDFAVYYCQQYNNWITFGQGTRLEIKRTVAAPSVFIFPPSDEQLKSGTASVVCLLNNFYPREAKVQWKVDNALQSGNSQESVTEQDSKDSTYSLSSTLTLSKADYEKHKVYACEVTHQGLSSPVTKSFNRGEC

SEQ ID NO: 208 - protein, 213 aa, synthetic construct
DIQMTQSPSTLSASVGDRVTITCRASQSFDNWLAWYQQKPGKAPKLLIYKASSLESGVPSRFSGSGSGTEFTLTISSLQPDDFATYYCQQYNSYSTFGQGTRLEIKRTVAAPSVFIFPPSDEQLKSGTASVVCLLNNFYPREAKVQWKVDNALQSGNSQESVTEQDSKDSTYSLSSTLTLSKADYEKHKVYACEVTHQGLSSPVTKSFNRGEC

SEQ ID NO: 209 - protein, 214 aa, synthetic construct
EIVMTQSPATLSVSPGERATLSCRASQSVSDTLAWYQQKPGQAPRLLIYGASTRATGIPARFSGSGSGTEFTLTISSLQSEDFAVYYCQQYNYWPLTFGGGTKVEIRRTVAAPSVFIFPPSDEQLKSGTASVVCLLNNFYPREAKVQWKVDNALQSGNSQESVTEQDSKDSTYSLSSTLTLSKADYEKHKVYACEVTHQGLSSPVTKSFNRGEC

SEQ ID NO: 210 - protein, 213 aa, synthetic construct
DFQMTQSPSTLSASVGDRVTITCRASQSISSWLAWYQQKPGKAPKLLIYEASSLKSGVPSRFSGSESGTEFTLTISSLQPDDFATYYCHQYNSYSTFGQGTKVEIKRTVAAPSVFIFPPSDEQLKSGTASVVCLLNNFYPREAKVQWKVDNALQSGNSQESVTEQDSKDSTYSLSSTLTLSKADYEKHKVYACEVTHQGLSSPVTKSFNRGEC

SEQ ID NO: 211 - protein, 213 aa, synthetic construct
DIQMTQSPSTLSASVGDRVTITCRASQSISSWLAWYQQKPGKAPKLLIYKASSLESGVPSRFSGSESGTEFTLTISSLQPDDFATYYCQQYNSYSTFGQGTKVEIKRTVAAPSVFIFPPSDEQLKSGTASVVCLLNNFYPREAKVQWKVDNALQSGNSQESVTEQDSKDSTYSLSSTLTLSKADYEKHKVYACEVTHQGLSSPVTKSFNRGEC

SEQ ID NO: 212 - protein, 213 aa, synthetic construct
DIQMTQSPSTLSASVGDRVTITCRASQSISSWLAWYQQKPGKAPKLLIYKASSLESGVPSRFSGSESGTEFTLTITSLQPNDFATYYCQQYNSYSTFGQGTRLEIKRTVAAPSVFIFPPSDEQLKSGTASVVCLLNNFYPREAKVQWKVDNALQSGNSQESVTEQDSKDSTYSLSSTLTLSKADYEKHKVYACEVTHQGLSSPVTKSFNRGEC

SEQ ID NO: 213 - protein, 214 aa, synthetic construct
EIVMTQSPATLSVSPGERATFSCRASQTVSSDLAWYQQKPGQAPRLLIYGASTRATGIPARFSGSGSGTEFTLTISSLQSEDFAFYYCQQSNDWPYTFGQGTKLEIKRTVAAPSVFIFPPSDEQLKSGTASVVCLLNNFYPREAKVQWKVDNALQSGNSQESVTEQDSKDSTYSLSSTLTLSKADYEKHKVYACEVTHQGLSSPVTKSFNRGEC

SEQ ID NO: 214 - protein, 213 aa, synthetic construct
DFQMTQSPSTLSASVGDRVTITCRASQSISSWLAWYQQKPGKAPKLLIYEASSLKSGVPSRFSGSESGTEFTLTISSLQPDDFATYYCHQYLSYSTFGQGTKVEIKRTVAAPSVFIFPPSDEQLKSGTASVVCLLNNFYPREAKVQWKVDNALQSGNSQESVTEQDSKDSTYSLSSTLTLSKADYEKHKVYACEVTHQGLSSPVTKSFNRGEC

SEQ ID NO: 215 - protein, 213 aa, synthetic construct
DFQMTQSPSTLSASVGDRVTITCRASQSISSWLAWYQQKPGKAPKLLIYEASSLKSGVPSRFSGSESGTEFTLTISSLQPDDFATYYCHQYMSYSTFGQGTKVEIKRTVAAPSVFIFPPSDEQLKSGTASVVCLLNNFYPREAKVQWKVDNALQSGNSQESVTEQDSKDSTYSLSSTLTLSKADYEKHKVYACEVTHQGLSSPVTKSFNRGEC

SEQ ID NO: 216 - protein, 219 aa, synthetic construct
DIVMTQSPLSLPVTPGEPASISCRSSQSLLHRDVYNYVDWYLQKPGQSPQLLIYLGSNRASGVPDRFSGSGSGTDFTLKISRVEAEDVGVYYCLQALQTPLTFGGGTKVEIKRTVAAPSVFIFPPSDEQLKSGTASVVCLLNNFYPREAKVQWKVDNALQSGNSQESVTEQDSKDSTYSLSSTLTLSKADYEKHKVYACEVTHQGLSSPVTKSFNRGEC

SEQ ID NO: 217 - protein, 446 aa, synthetic construct
QVQLVQSGAEVKKPGSSVKVSCKASGYTFTSYRMHWVRQAPGQGLEWIGYINPSTGYTEYNQKFKDKATITADESTNTAYMELSSLRSEDTAVYYCARGGGVFDYWGQGTLVTVSSASTKGPSVFPLAPSSKSTSGGTAALGCLVKDYFPEPVTVSWNSGALTSGVHTFPAVLQSSGLYSLSSVVTVPSSSLGTQTYICNVNHKPSNTKVDKKVEPKSCDKTHTCPPCPAPELLGGPSVFLFPPKPKDTLMISRTPEVTCVVVDVSHEDPEVKFNWYVDGVEVHNAKTKPREEQYNSTYRVVSVLTVLHQDWLNGKEYKCKVSNKALPAPIEKTISKAKGQPREPQVYTLPPSRDELTKNQVSLTCLVKGFYPSDIAVEWESNGQPENNYKTTPPVLDSDGSFFLYSKLTVDKSRWQQGNVFSCSVMHEALHNHYTQKSLSLSPGK

SEQ ID NO: 218 - protein, 213 aa, synthetic construct
DIQMTQSPSTLSASVGDRVTITCSASSSISYMHWYQQKPGKAPKLLIYTTSNLASGVPARFSGSGSGTEFTLTISSLQPDDFATYYCHQRSTYPLTFGQGTKVEVKRTVAAPSVFIFPPSDEQLKSGTASVVCLLNNFYPREAKVQWKVDNALQSGNSQESVTEQDSKDSTYSLSSTLTLSKADYEKHKVYACEVTHQGLSSPVTKSFNRGEC